European Patent Application EP 4 624 498 A1, published October 1, 2025. Title: 一种融合多肽及其用途. Applicant: 苏州沙砾生物科技有限公司. Application WO. The sequence listing filed with the application follows.

SEQUENCE LISTING (62 sequences)

SEQ ID NO: 1 - protein, 22 aa, synthetic construct
VAISTTVLLCGLSAVSLLACYL

SEQ ID NO: 2 - protein, 22 aa, synthetic construct
VASTSTVLLCGLSAVSLLACYL

SEQ ID NO: 3 - protein, 22 aa, synthetic construct
VAITSTVLLCGLSAVSLLACYL

SEQ ID NO: 4 - protein, 22 aa, synthetic construct
VAISSTVLLCGLSAVSLLACYL

SEQ ID NO: 5 - protein, 29 aa, synthetic construct
MRISKPHLRSISIQCYLCLLLNSHFLTEA

SEQ ID NO: 6 - protein, 28 aa, synthetic construct
MVAGSDAGRALGVLSVVCLLHCFGFISC

SEQ ID NO: 7 - protein, 31 aa, synthetic construct
SGGGSGGGGSGGGGSGGGGSGGGGSGGGSLQ

SEQ ID NO: 8 - protein, 36 aa, synthetic construct
SGGGSGGGGSGGGGSGGGGSGGGGSGGGGSGGGSLQ

SEQ ID NO: 9 - protein, 394 aa, synthetic construct
MDWTWILFLVAAATRVHSNWVNVISDLKKIEDLIQSMHIDATLYTESDVHPSCKVTAMKCFLLELQVISLESGDASIHDTVENLIILANNSLSSNGNVTESGCKECEELEEKNIKEFLQSFVHIVQMFINTSSGGGSGGGGSGGGGSGGGGSGGGSLQITCPPPMSVEHADIWVKSYSLYSRERYICNSGFKRKAGTSSLTECVLNKATNVAHWTTPSLKCIRDPALVHQRPAPPSTVTTAGVTPQPESLSPSGKEPAASSPSSNNTAATTAAIVPGSQLMPSKSPSTGTTEISSHESSHGTPSQTTAKNWELTASASHQPPGVYPQGHSDTTVAISTTVLLCGLSAVSLLACYLKSRQTPPLASVEMEAMEALPVTWGTSSRDEDLENCSHHL

SEQ ID NO: 10 - protein, 18 aa, synthetic construct
MDWTWILFLVAAATRVHS

SEQ ID NO: 11 - protein, 114 aa, synthetic construct
NWVNVISDLKKIEDLIQSMHIDATLYTESDVHPSCKVTAMKCFLLELQVISLESGDASIHDTVENLIILANNSLSSNGNVTESGCKECEELEEKNIKEFLQSFVHIVQMFINTS

SEQ ID NO: 12 - protein, 26 aa, synthetic construct
SGGGSGGGGSGGGGSGGGGSGGGSLQ

SEQ ID NO: 13 - protein, 175 aa, synthetic construct
ITCPPPMSVEHADIWVKSYSLYSRERYICNSGFKRKAGTSSLTECVLNKATNVAHWTTPSLKCIRDPALVHQRPAPPSTVTTAGVTPQPESLSPSGKEPAASSPSSNNTAATTAAIVPGSQLMPSKSPSTGTTEISSHESSHGTPSQTTAKNWELTASASHQPPGVYPQGHSDTT

SEQ ID NO: 14 - protein, 23 aa, synthetic construct
  SITE 3: note = misc_feature - Xaa = Ile or missing
  SITE 4: note = misc_feature - Xaa = Ser or missing
  SITE 5: note = misc_feature - Xaa = Thr or missing
  SITE 6: note = misc_feature - Xaa = Ser or missing
VAXXXXTVLLCGLSAVSLLACYL

SEQ ID NO: 15 - protein, 39 aa, synthetic construct
KSRQTPPLASVEMEAMEALPVTWGTSSRDEDLENCSHHL

SEQ ID NO: 16 - protein, 395 aa, synthetic construct [sequence omitted]

SEQ ID NO: 17 - protein, 23 aa, synthetic construct
VAISTSTVLLCGLSAVSLLACYL

SEQ ID NO: 18 - protein, 394 aa, synthetic construct
MDWTWILFLVAAATRVHSNWVNVISDLKKIEDLIQSMHIDATLYTESDVHPSCKVTAMKCFLLELQVISLESGDASIHDTVENLIILANNSLSSNGNVTESGCKECEELEEKNIKEFLQSFVHIVQMFINTSSGGGSGGGGSGGGGSGGGGSGGGSLQITCPPPMSVEHADIWVKSYSLYSRERYICNSGFKRKAGTSSLTECVLNKATNVAHWTTPSLKCIRDPALVHQRPAPPSTVTTAGVTPQPESLSPSGKEPAASSPSSNNTAATTAAIVPGSQLMPSKSPSTGTTEISSHESSHGTPSQTTAKNWELTASASHQPPGVYPQGHSDTTVASTSTVLLCGLSAVSLLACYLKSRQTPPLASVEMEAMEALPVTWGTSSRDEDLENCSHHL

SEQ ID NO: 19 - protein, 394 aa, synthetic construct
MDWTWILFLVAAATRVHSNWVNVISDLKKIEDLIQSMHIDATLYTESDVHPSCKVTAMKCFLLELQVISLESGDASIHDTVENLIILANNSLSSNGNVTESGCKECEELEEKNIKEFLQSFVHIVQMFINTSSGGGSGGGGSGGGGSGGGGSGGGSLQITCPPPMSVEHADIWVKSYSLYSRERYICNSGFKRKAGTSSLTECVLNKATNVAHWTTPSLKCIRDPALVHQRPAPPSTVTTAGVTPQPESLSPSGKEPAASSPSSNNTAATTAAIVPGSQLMPSKSPSTGTTEISSHESSHGTPSQTTAKNWELTASASHQPPGVYPQGHSDTTVAITSTVLLCGLSAVSLLACYLKSRQTPPLASVEMEAMEALPVTWGTSSRDEDLENCSHHL

SEQ ID NO: 20 - protein, 394 aa, synthetic construct
MDWTWILFLVAAATRVHSNWVNVISDLKKIEDLIQSMHIDATLYTESDVHPSCKVTAMKCFLLELQVISLESGDASIHDTVENLIILANNSLSSNGNVTESGCKECEELEEKNIKEFLQSFVHIVQMFINTSSGGGSGGGGSGGGGSGGGGSGGGSLQITCPPPMSVEHADIWVKSYSLYSRERYICNSGFKRKAGTSSLTECVLNKATNVAHWTTPSLKCIRDPALVHQRPAPPSTVTTAGVTPQPESLSPSGKEPAASSPSSNNTAATTAAIVPGSQLMPSKSPSTGTTEISSHESSHGTPSQTTAKNWELTASASHQPPGVYPQGHSDTTVAISSTVLLCGLSAVSLLACYLKSRQTPPLASVEMEAMEALPVTWGTSSRDEDLENCSHHL

SEQ ID NO: 21 - protein, 18 aa, synthetic construct
MDWTWILFLVAAATRVHS

SEQ ID NO: 22 - protein, 29 aa, synthetic construct
MRISKPHLRSISIQCYLCLLLNSHFLTEA

SEQ ID NO: 23 - protein, 28 aa, synthetic construct
MVAGSDAGRALGVLSVVCLLHCFGFISC

SEQ ID NO: 24 - protein, 114 aa, synthetic construct; identical to SEQ ID NO: 11

SEQ ID NO: 25 - protein, 26 aa, synthetic construct
SGGGSGGGGSGGGGSGGGGSGGGSLQ

SEQ ID NO: 26 - protein, 26 aa, synthetic construct
KESGSVSSEQLAQFRSLDSGSESKST

SEQ ID NO: 27 - protein, 26 aa, synthetic construct
KESGSVSSEQLAQFRSLDSAAGSGEF

SEQ ID NO: 28 - protein, 26 aa, synthetic construct
GEDSTAPGEDSTAPGSAGSAAGSGEF

SEQ ID NO: 29 - protein, 26 aa, synthetic construct
GQAPKESGSVSSEQLAQFRSLDGQAP

SEQ ID NO: 30 - protein, 26 aa, synthetic construct
SSEQLAQFRSLDEGKSSGSGSESKST

SEQ ID NO: 31 - protein, 26 aa, synthetic construct
SGSESKSTKESGSVSSEQLAQFRSLD

SEQ ID NO: 32 - protein, 26 aa, synthetic construct
SAAGSGEFKESGSVSSEQLAQFRSLD

SEQ ID NO: 33 - protein, 26 aa, synthetic construct
GEDSTAPGQAPGQAPGQAPGEDSTAP

SEQ ID NO: 34 - protein, 26 aa, synthetic construct
KESGSVSSEQLAQFRSLDGEDSTAPG

SEQ ID NO: 35 - protein, 26 aa, synthetic construct
GEDSTAPGSAGSAAGSGEFGEDSTAP

SEQ ID NO: 36 - protein, 26 aa, synthetic construct
GQAPGQAPKESGSVSSEQLAQFRSLD

SEQ ID NO: 37 - protein, 26 aa, synthetic construct
GQAPKESGSVSSEQLAQFRSLDSGGS

SEQ ID NO: 38 - protein, 26 aa, synthetic construct
GQAPGPASGEDSTAPGEDSTAPGQAP

SEQ ID NO: 39 - protein, 25 aa, synthetic construct
KESGSVSSEQLAQFRSLDGEDSTAP

SEQ ID NO: 40 - protein, 32 aa, synthetic construct
KESGSVSSEQLAQFRSLDEGKSSGSGSESKST

SEQ ID NO: 41 - protein, 30 aa, synthetic construct
KESGSVSSEQLAQFRSLDGSAGSAAGSGEF

SEQ ID NO: 42 - protein, 22 aa, synthetic construct
KESGSVSSEQLAQFRSLDGQAP

SEQ ID NO: 43 - protein, 26 aa, synthetic construct
EGKSSGSGSESKSTGSAGSAAGSGEF

SEQ ID NO: 44 - protein, 30 aa, synthetic construct
EGKSSGSGSESKSTGQAPGSAGSAAGSGEF

SEQ ID NO: 45 - protein, 25 aa, synthetic construct
EGKSSGSGSESKSTGEDSTAPGQAP

SEQ ID NO: 46 - protein, 24 aa, synthetic construct
EGKSSGSGSESKSTPASGQAPPAS

SEQ ID NO: 47 - protein, 24 aa, synthetic construct
EGKSSGSGSESKSTPASGEDSTAP

SEQ ID NO: 48 - protein, 21 aa, synthetic construct
KESGSVSSEQLAQFRSLDPAS

SEQ ID NO: 49 - protein, 175 aa, synthetic construct; identical to SEQ ID NO: 13

SEQ ID NO: 50 - protein, 23 aa, synthetic construct
  SITE 3: note = misc_feature - Xaa = Ile or missing
  SITE 4: note = misc_feature - Xaa = Ser or missing
  SITE 5: note = misc_feature - Xaa = Thr or missing
  SITE 6: note = misc_feature - Xaa = Ser or missing
VAXXXXTVLLCGLSAVSLLACYL

SEQ ID NO: 51 - protein, 22 aa, synthetic construct
VAISTTVLLCGLSAVSLLACYL

SEQ ID NO: 52 - protein, 22 aa, synthetic construct
VASTSTVLLCGLSAVSLLACYL

SEQ ID NO: 53 - protein, 22 aa, synthetic construct
VAITSTVLLCGLSAVSLLACYL

SEQ ID NO: 54 - protein, 22 aa, synthetic construct
VAISSTVLLCGLSAVSLLACYL

SEQ ID NO: 55 - protein, 23 aa, synthetic construct
VAISTSTVLLCGLSAVSLLACYL

SEQ ID NO: 56 - protein, 39 aa, synthetic construct; identical to SEQ ID NO: 15

SEQ ID NO: 57 - protein, 395 aa, synthetic construct [sequence omitted]

SEQ ID NO: 58 - protein, 394 aa, synthetic construct; identical to SEQ ID NO: 9

SEQ ID NO: 59 - protein, 405 aa, synthetic construct
MRISKPHLRSISIQCYLCLLLNSHFLTEANWVNVISDLKKIEDLIQSMHIDATLYTESDVHPSCKVTAMKCFLLELQVISLESGDASIHDTVENLIILANNSLSSNGNVTESGCKECEELEEKNIKEFLQSFVHIVQMFINTSKESGSVSSEQLAQFRSLDSAAGSGEFITCPPPMSVEHADIWVKSYSLYSRERYICNSGFKRKAGTSSLTECVLNKATNVAHWTTPSLKCIRDPALVHQRPAPPSTVTTAGVTPQPESLSPSGKEPAASSPSSNNTAATTAAIVPGSQLMPSKSPSTGTTEISSHESSHGTPSQTTAKNWELTASASHQPPGVYPQGHSDTTVAISTTVLLCGLSAVSLLACYLKSRQTPPLASVEMEAMEALPVTWGTSSRDEDLENCSHHL

SEQ ID NO: 60 - protein, 404 aa, synthetic construct
MVAGSDAGRALGVLSVVCLLHCFGFISCNWVNVISDLKKIEDLIQSMHIDATLYTESDVHPSCKVTAMKCFLLELQVISLESGDASIHDTVENLIILANNSLSSNGNVTESGCKECEELEEKNIKEFLQSFVHIVQMFINTSKESGSVSSEQLAQFRSLDSAAGSGEFITCPPPMSVEHADIWVKSYSLYSRERYICNSGFKRKAGTSSLTECVLNKATNVAHWTTPSLKCIRDPALVHQRPAPPSTVTTAGVTPQPESLSPSGKEPAASSPSSNNTAATTAAIVPGSQLMPSKSPSTGTTEISSHESSHGTPSQTTAKNWELTASASHQPPGVYPQGHSDTTVAISTTVLLCGLSAVSLLACYLKSRQTPPLASVEMEAMEALPVTWGTSSRDEDLENCSHHL

SEQ ID NO: 61 - protein, 405 aa, synthetic construct
MRISKPHLRSISIQCYLCLLLNSHFLTEANWVNVISDLKKIEDLIQSMHIDATLYTESDVHPSCKVTAMKCFLLELQVISLESGDASIHDTVENLIILANNSLSSNGNVTESGCKECEELEEKNIKEFLQSFVHIVQMFINTSGQAPKESGSVSSEQLAQFRSLDGQAPITCPPPMSVEHADIWVKSYSLYSRERYICNSGFKRKAGTSSLTECVLNKATNVAHWTTPSLKCIRDPALVHQRPAPPSTVTTAGVTPQPESLSPSGKEPAASSPSSNNTAATTAAIVPGSQLMPSKSPSTGTTEISSHESSHGTPSQTTAKNWELTASASHQPPGVYPQGHSDTTVAISTTVLLCGLSAVSLLACYLKSRQTPPLASVEMEAMEALPVTWGTSSRDEDLENCSHHL

SEQ ID NO: 62 - protein, 404 aa, synthetic construct
MVAGSDAGRALGVLSVVCLLHCFGFISCNWVNVISDLKKIEDLIQSMHIDATLYTESDVHPSCKVTAMKCFLLELQVISLESGDASIHDTVENLIILANNSLSSNGNVTESGCKECEELEEKNIKEFLQSFVHIVQMFINTSGQAPKESGSVSSEQLAQFRSLDGQAPITCPPPMSVEHADIWVKSYSLYSRERYICNSGFKRKAGTSSLTECVLNKATNVAHWTTPSLKCIRDPALVHQRPAPPSTVTTAGVTPQPESLSPSGKEPAASSPSSNNTAATTAAIVPGSQLMPSKSPSTGTTEISSHESSHGTPSQTTAKNWELTASASHQPPGVYPQGHSDTTVAISTTVLLCGLSAVSLLACYLKSRQTPPLASVEMEAMEALPVTWGTSSRDEDLENCSHHL